European Patent Specification EP 3 373 723 B1, published August 20, 2025. Title: Resistance to ToLCNDV in Squash. Applicant: Vilmorin and Cie Aguilar, Juan Justafre, Isabelle Lionneton, Eric Mazet, Julien. The sequence listing filed with the application follows.

SEQUENCE LISTING (10 sequences)

SEQ ID NO: 1 - DNA, 2738 bp, Tomato Leaf Curl New Delhi Virus
accgaatggccgcgaaattttttggtgggccctgaaccaatagaattcaagttacatggcttatttagtgcgtggggaccaataaatagacttgctcaccaagtttagatccacaaacatgtgggatccattattgcacgaatttccggaaagcgtccatggtctaaggtgcatgttagctgtaaaatatctccaagagattgagaagtcctattctccagacacagtcggctacgatcttgtccgagatctcattttagttctccgagccaagaactatgtcgaagcgaccagcagatatcatcatttcaactcccgcatcgaaggtacgccgacggctcaacttcgacagcccctatggaacccgtgcctctgtccccattgcccgcgtcacaaaagcaagggcctggacgaacaggcccatgaacagaaaacccagaatgtacagaatgtatagaagtcctgacgtgccaaggggttgtgaaggcccttgtaaggtgcaatcgtttgaatcccggcacgatgtctcgcatattggcaaagtcatgtgtgttagtgatgttactcgaggcaccggactcacacatcgcgtaggcaagcgattttgtgtgaaatctgtctatgtactgggaaaaatatggatggatgaaaatatcaaaactaaaaatcatactaatagtgttatgttctttcttgttcgtgaccggcgtccaaccggaacccctcaagattttggggaagttttcaatatgtttgataatgaacctagcacagccacggtgaagaacatgcatcgtgatcgttatcaagtcttacggaagtggcatgctactgtgacgggaggaacgtatgcatcaagggagcaagcattagttaggaagtttgttagggttaataattatgttgtttacaatcaacaagaggccggcaagtatgagaatcatactgaaaatgcattaatgttgtatatggcctgtactcatgcatcaaatcctgtgtatgctactttgaaaatccggatctatttttatgattcggtcacaaattaatatatattgatctttacatcatatgttgtccatacatcaatcgttttatgcaagacattatctaaaacatgataaacagctcttattacattacaaatgccgactacaccaagcatatttaggtacttaaggacctgcgttctaaaaaccctcaagaaaatcccagtcggagggcgtaagcccgtccagatttggaaagttagaaaacacttgtgaagccccagagctttccgcaggttgtggttgaactgtacttggactttgattatgtcgtgattggtcaggcacggtctgctgtcgtgtttcaatactttgaaatacaggggatttggtacgtcccagataaagacgccactctcttctcgatccgcagtgatgtactcccctgtgcgtgaatccgtgatcatggcaattgatcgatatgtagtaggaacaaccgcactgcagatcaactcgcctcctgcgaatgttcttcttcttcttctgggggagcgatgttttcgcgactggaatagagtggttcttcgagtgtgatgaagactgcattcttgattgcccactgcttcagtgctgcatttttttcttcgtcaagatattctttataactgctgtttggtccttcattgcacaggaagatagtgggaattccacctttaatcatgacaggctttccgtacttcgtgttgctttgccagtcacgttgggcccccatgaattctttaaaatgctttagatagtggggatcaacgtcgtcaatgacgttgtaccaggcatcattgctataaacttttgggctaagatccagatgaccacacaaataattgtggggtcctaaacaacgcgcccacattgttttgcccgtcctactatcgccctgtatgactatgcttattggtcttaaaggccgcgcagckgaacacaccacattacatttggcccaatcgacgagatctgcaggaactctgtcgaaggatgaaatcgaaaaaggagaaacataaacctccgaacgagtctggaaaatgcgatctaaattattaattaaattatgaaactgcagaacataatcttttggtgctagttcctttaaaacctttaacgcatctgtcttgtttccagtgttaattgcctgagcatatgcatcgttggccgtttgttgaccaccacgagcagatcgtccatcgatctgaaaaacaccccattctagaacgtctccgtctttgtcgatgtatgccttgacgtccgacgctgatttagctccctgaatgttcggatggaaatgtgctgccctacttggggacaccaagtcgaagaatctgttattcttgcactggaatttcccttcgaattggacgagaacatggatatgcggagacccatcctcgtgaagctctctacagatcttgatgaatttcttcgaagttggggtttctagggtttgtaattgggaaagtgcctcttcctttgtaagagagcacttcggatacgtgaggaaatagtttttggcatttattctaaaacgacttggcggagccataaaaagtgtcgtttcgatctggtgtctctcaacttcctgtatgtaattggtgtctggagtcccatatataggtaagacactaaatggcagaattgtaattttgaagagaaaattactttaaatcaaatttcaaaagcggccattcgtataatatt

SEQ ID NO: 2 - DNA, 2738 bp, Tomato Leaf Curl New Dehli Virus
accgaatggccgcgaaattttttggtgggccctgaaccaatagaattcaagttacatggcttatttagtgcgtggggaccaataaatagacttgctcaccaagtttagatccacaaacatgtgggatccattattgcacgaatttccggaaagcgtccatggtctaaggtgcatgttagctgtaaaatatctccaagagattgagaagtcctattctccagacacagtcggctacgatcttgtccgagatctcattttagttctccgagccaagaactatgtcgaagcgaccagcagatatcatcatttcaactcccgcatcgaaggtacgccgacggctcaacttcgacagcccctatggaacccgtgcctctgtccccattgcccgcgtcacaaaagcaagggcctggacgaacaggcccatgaacagaaaacccagaatgtacagaatgtatagaagtcctgacgtgccaaggggttgtgaaggcccttgtaaggtgcaatcgtttgaatcccggcacgatgtctcgcatattggcaaagtcatgtgtgttagtgatgttactcgaggcaccggactcacacatcgcgtaggcaagcgattttgtgtgaaatctgtctatgtactgggaaaaatatggatggatgaaaatatcaaaactaaaaatcatactaatagtgttatgttctttcttgttcgtgaccggcgtccaaccggaacccctcaagattttggggaagttttcaatatgtttgataatgaacctagcacagccacggtgaagaacatgcatcgtgatcgttatcaagtcttacggaagtggcatgctactgtgacgggaggaacgtatgcatcaagggagcaagcattagttaggaagtttgttagggttaataattatgttgtttacaatcaacaagaggccggcaagtatgagaatcatactgaaaatgcattaatgttgtatatggcctgtactcatgcatcaaatcctgtgtatgctactttgaaaatccggatctatttttatgattcggtcacaaattaatatatattgatctttacatcatatgttgtccatacatcaatcgttttatgcaagacattatctaaaacatgataaacagctcttattacattacaaatgccgactacaccaagcatatttaggtacttaaggacctgcgttctaaaaaccctcaagaaaatcccagtcggagggcgtaagcccgtccagatatggaaagttagaaaacacttgtgaagccccagagctttccgcaggttgtggttgaactgtacttggattttgattatgtcgtgattggtcaggcacggtctgctgtcgtgtttcaatactttgaaatacaggggatttggtacgtcccagataaagacgccactctctgctcgatccgcagtgatgtactcccctgtgcgtgaatccgtgatcatggcaattgatcgatatgtagtaggaacaaccgcactgcagatcaactcgcctcctgcgaatgttcttcttcttcttctgggggagcgatgttttcgcgactggaatagagtggttcttcgagtgtgatgaagactgcattcttgattgcccactgcttcagtgctgcatttttttcttcgtcaagatattctttataactgctgtttggtccttcattgcacaggaagatagtgggaattccacctttaatcatgacaggctttccgtactttgtgttgctttgccagtcacgttgggcccccatgaattctttaaagtgctttagatagtggggatcaacgtcgtcaatgacgttgtaccaggcatcattgctataaacttttgggctaagatccagatgaccacacaaataattgtggggtcctaaacaacgcgcccacattgttttgcccgtcctactatctccctctatgactatgcttattggtcttaatggccgcgcagcggaacacaccacattacatttggcccaatcgacgagatctgcaggaactctgtcgaaggatgaaatcgaaaaaggagaaacataaacctccgaacgagtctggaaaatgcgatctaaattattaattaaattatgaaactgcagaacataatcttttggtgctagttcctttaaaacctttaacgcatctgtcttgtttccagtgttaattgcctgagcatatgcatcgttggccgtttgttgaccaccacgagcagatcgtccatcgatctgaaaaacaccccattctagaacgtctccgtctttgtcgatgtatgtcttgacgtccgacgctgatttagctccctgaatgttcggatggaaatgtgctgccctacttggggacaccaagtcgaagaatctgttattcttgcactggaatttcccttcgaattggacgagaacatggatatgcggagacccatcctcgtgaagctctctacagatcttgatgaatttcttcgaagttggggtttctagggtttgtaattgggaaagtgcctcttcctttgtaagagagcacttcggatacgtgaggaaatagttttttgcatttattctaaaacgacttggcggagccataaaacgtgtcgtttcgatctggtgtctctcaacttcctgtatgtaattggtgtctggagtcccatatataggtaagacactaaatggcagaattgtaattttgaagagaaaattactttaattcaaatttcaaaagcggccattcgtataatatt

SEQ ID NO: 3 - DNA, 970 bp, Tomato Leaf Curl New Dehli Virus
tttggctgtgaaaggcccatgtaaggtgcaatcgtttgaatcccggcacgatgtctcgcatattggcaaagtcatgtgtgttagtgatgttactcgaggcaccggactcacacatcgcgtaggcaagcgattttgtgtgaaatctgtctatgtactgggaaaaatatggatggatgaaaatatcaaaactaaaaatcatactaatagtgttatgttctttcttgttcgtgaccggcgtccaaccggaacccctcaagattttggggaagttttcaatatgtttgataatgaacctagcacagccacggtgaagaacatgcatcgtgatcgttatcaagtcttacggaagtggcatgctactgtgacgggaggaacgtatgcatcaagggagcaagcattagttaggaagtttgttagggttaataattatgttgtttacaatcaacaagaggccggcaagtatgagaatcatactgaaaatgcattaatgttgtatatggcctgtactcatgcatcaaatcctgtgtatgctactttgaaaatccggatctatttttatgattcggtcacaaattaatatatattgatctttacatcatatgttgtccatacatcaatcgttttatgcaagacattatctaaaacatgataaacagctcttattacattacaaatgccgactacaccaagcatatttaggtacttaaggacctgcgttctaaaaaccctcaagaaaatcccagtcggagggcgtaagcccgtccagatttggaaagttagaaaacacttgtgaagccccagagctttccgcaggttgtggttgaactgtacttggactttgattatgtcgtgattggtcaggcacggtctgctgtcgtgtttcaatactttgaaatacaggggatttggtacgtcccagataaagacgccactctctgctcgatccgcagtgatgtactcccctgtgcgt

SEQ ID NO: 4 - DNA, 20 bp, Unknown
  Forward primer
ggctgtgaaggcccatgtaa

SEQ ID NO: 5 - DNA, 19 bp, Unknown
  Reverse primer
atggattcacgcacagggg

SEQ ID NO: 6 - DNA, 23 bp, Unknown
  Forward primer
ttggatccatggcgaagcgacca

SEQ ID NO: 7 - DNA, 23 bp, Unknown
  Reverse primer
aagagctcttaatttgtgaccga

SEQ ID NO: 8 - DNA, 71 bp, Unknown
  Flanking sequence of marker SQ-0006678
  misc_feature (1)..(71): allele G: Resistant allele
  misc_feature (1)..(71): allele A: Susceptible allele
gttgtaagtccagcaatagcaccaacgcttatcaaraaagaaacaaatttcaagcctttggatgtaaaagc

SEQ ID NO: 9 - DNA, 71 bp, Unknown
  Flanking sequence of marker SQ-0010844
  misc_feature (1)..(71): allele G: Resistant allele
  misc_feature (1)..(71): allele A: Susceptible allele
aaaagagaaagttggaggactgagttgccaagggcmggcctgggatctgaagtcattgtgaaaatgaaaaa

SEQ ID NO: 10 - DNA, 155 bp, Unknown
  Flanking sequence of marker SQ-0000209
  misc_feature (86)..(86): n is a, c, g, or t
  misc_feature (91)..(91): n is a, c, g, or t
  misc_feature (1)..(155): allele G: Resistant allele
  misc_feature (1)..(155): allele A: Susceptible allele
ttaacaccaccgattctcagctccagtagcaagaccagtagactgccatggaactccatcgttctcagaggaaatcttccaccgcnaccanttcctcgaccactcttccactctatcgctcmgctcctcctctcgaagtcaggcttgaagaattc